European Patent Application EP 4 289 860 A1, published December 13, 2023. Title: A use of a Polypeptide Compound in the Preparation of Drugs for Preventing or Treating Inflammatory Bowel Diseases and Related Intestinal Fibrosis. Applicant: Shenzhen Turier Biotech Co., Ltd. The sequence listing filed with the application follows.

SEQUENCE LISTING (16 sequences)

SEQ ID NO: 1 - protein, 39 aa, Artificial Sequence
  Compound 1
  MISC_FEATURE (2)..(2): X=Aib
  MISC_FEATURE (10)..(10): A side chain of Lys is linked to -PEG2-PEG2-γGlu-CO(CH2)18CO2H
  MISC_FEATURE (16)..(16): X=Aib
HXQGTFTSDKSKYLEXKAAQDFVEWLKAGGPSSGAPPPS

SEQ ID NO: 2 - protein, 39 aa, Artificial Sequence; identical to SEQ ID NO: 1
  Compound 2
  MISC_FEATURE (2)..(2): X=D-Ser
  MISC_FEATURE (10)..(10): A side chain of Lys is linked to -PEG2-PEG2-CO(CH2)18CO2H
  MISC_FEATURE (16)..(16): X=Aib

SEQ ID NO: 3 - protein, 39 aa, Artificial Sequence; identical to SEQ ID NO: 1
  Compound 3
  MISC_FEATURE (2)..(2): X=D-Ser
  MISC_FEATURE (10)..(10): A side chain of Lys is linked to -PEG2-PEG2-γGlu-CO(CH2)18CO2H
  MISC_FEATURE (16)..(16): X=Aib

SEQ ID NO: 4 - protein, 39 aa, Artificial Sequence; identical to SEQ ID NO: 1
  Compound 4
  MISC_FEATURE (2)..(2): X=D-Ser
  MISC_FEATURE (10)..(10): A side chain of Lys is linked to -PEG2-PEG2-γGlu-CO(CH2)16CO2H
  MISC_FEATURE (16)..(16): X=Aib

SEQ ID NO: 5 - protein, 39 aa, Artificial Sequence; identical to SEQ ID NO: 1
  Compound 5
  MISC_FEATURE (2)..(2): X=D-Ser
  MISC_FEATURE (10)..(10): A side chain of Lys is linked to -PEG2-PEG2-γGlu-CO(CH2)18CH3
  MISC_FEATURE (16)..(16): X=Aib

SEQ ID NO: 6 - protein, 39 aa, Artificial Sequence
  Compound 6
  MISC_FEATURE (2)..(2): X=D-Ser
  MISC_FEATURE (10)..(10): A side chain of Lys is linked to -PEG2-PEG2-γGlu-CO(CH2)18CO2H
  MISC_FEATURE (23)..(23): X=Isovaline
  MISC_FEATURE (35)..(35): X=Aib
HXQGTFTSDKSKYLDERAAQDFXQWLLDGGPSSGXPPPS

SEQ ID NO: 7 - protein, 39 aa, Artificial Sequence
  Compound 7
  MISC_FEATURE (2)..(2): X=D-Ser
  MISC_FEATURE (10)..(10): A side chain of Lys is linked to -PEG2-PEG2-γGlu-CO(CH2)18CO2H
  MISC_FEATURE (23)..(23): X=Isovaline
HXQGTFTSDKSKYLDERAAQDFXQWLLEGGPSSGAPPPS

SEQ ID NO: 8 - protein, 39 aa, Artificial Sequence; identical to SEQ ID NO: 6
  Compound 8
  MISC_FEATURE (2)..(2): X=Aib
  MISC_FEATURE (10)..(10): A side chain of Lys is linked to -PEG2-PEG2-γGlu-CO(CH2)18CO2H
  MISC_FEATURE (23)..(23): X=Isovaline
  MISC_FEATURE (35)..(35): X=Aib

SEQ ID NO: 9 - protein, 39 aa, Artificial Sequence; identical to SEQ ID NO: 6
  Compound 9
  MISC_FEATURE (2)..(2): X=Aib
  MISC_FEATURE (10)..(10): A side chain of Lys is linked to -PEG2-PEG2-γGlu-CO(CH2)16CO2H
  MISC_FEATURE (23)..(23): X=Isovaline
  MISC_FEATURE (35)..(35): X=Aib

SEQ ID NO: 10 - protein, 39 aa, Artificial Sequence; identical to SEQ ID NO: 6
  Compound 10
  MISC_FEATURE (2)..(2): X=Aib
  MISC_FEATURE (10)..(10): A side chain of Lys is linked to -PEG2-PEG2-γGlu-CO(CH2)18CH3
  MISC_FEATURE (23)..(23): X=Isovaline
  MISC_FEATURE (35)..(35): X=Aib

SEQ ID NO: 11 - protein, 39 aa, Artificial Sequence; identical to SEQ ID NO: 6
  Compound 11
  MISC_FEATURE (2)..(2): X=Aib
  MISC_FEATURE (10)..(10): A side chain of Lys is linked to -PEG2-PEG2-γGlu-CO(CH2)18CH3
  MISC_FEATURE (23)..(23): X=Isovaline
  MISC_FEATURE (35)..(35): X=Aib

SEQ ID NO: 12 - protein, 39 aa, Artificial Sequence; identical to SEQ ID NO: 6
  Compound 12
  MISC_FEATURE (2)..(2): X=D-Ser
  MISC_FEATURE (10)..(10): A side chain of Lys is linked to -PEG2-PEG2-γGlu-CO(CH2)18CO2H
  MISC_FEATURE (23)..(23): X=Isovaline
  MISC_FEATURE (35)..(35): X=Aib

SEQ ID NO: 13 - protein, 39 aa, Artificial Sequence; identical to SEQ ID NO: 1
  Compound 13
  MISC_FEATURE (2)..(2): X=D-Ser
  MISC_FEATURE (10)..(10): A side chain of Lys is linked to -Gly-Gly-Ser-Gly-Ser-Gly-γGlu-CO(CH2)18-COOH
  MISC_FEATURE (16)..(16): X=Aib

SEQ ID NO: 14 - protein, 39 aa, Artificial Sequence; identical to SEQ ID NO: 1
  Compound 14
  MISC_FEATURE (2)..(2): X=D-Ser
  MISC_FEATURE (10)..(10): A side chain of Lys is linked to -Gly-Gly-Ser-Gly-Ser-Gly-γGlu-CO(CH2)18-COOH
  MISC_FEATURE (16)..(16): X=Aib

SEQ ID NO: 15 - protein, 39 aa, Artificial Sequence; identical to SEQ ID NO: 6
  Compound 15
  MISC_FEATURE (2)..(2): X=Aib
  MISC_FEATURE (10)..(10): A side chain of Lys is linked to -Gly-Gly-Ser-Gly-Ser-Gly-γGlu-CO(CH2)18-COOH
  MISC_FEATURE (23)..(23): X=Isovaline
  MISC_FEATURE (35)..(35): X=Aib

SEQ ID NO: 16 - protein, 39 aa, Artificial Sequence; identical to SEQ ID NO: 6
  Compound 16
  MISC_FEATURE (2)..(2): X=Aib
  MISC_FEATURE (10)..(10): A side chain of Lys is linked to -Gly-Gly-Ser-Gly-Ser-Gly-γGlu-CO(CH2)18-COOH
  MISC_FEATURE (23)..(23): X=Isovaline
  MISC_FEATURE (35)..(35): X=Aib